European Patent Application EP 4 471 066 A1, published December 4, 2024. Title: Antibody specifically binding to MUC-1 and uses thereof. Applicant: Cyron Therapeutics Co., Ltd. The sequence listing filed with the application follows.

SEQUENCE LISTING (115 sequences)

SEQ ID NO: 1 - protein, 5 aa, Artificial Sequence
  synthetic_VH-CDR1
  MOD_RES (1): Xaa is Asp or Ser
  MOD_RES (5): Xaa is Asn, Ser, or His
XYWMX

SEQ ID NO: 2 - protein, 5 aa, Artificial Sequence
  synthetic_VH-CDR1
DYWMN

SEQ ID NO: 3 - protein, 5 aa, Artificial Sequence
  synthetic_VH-CDR1
DYWMS

SEQ ID NO: 4 - protein, 5 aa, Artificial Sequence
  synthetic_VH-CDR1
SYWMN

SEQ ID NO: 5 - protein, 5 aa, Artificial Sequence
  synthetic_VH-CDR1
SYWMS

SEQ ID NO: 6 - protein, 5 aa, Artificial Sequence
  synthetic_VH-CDR1
SYWMH

SEQ ID NO: 7 - protein, 19 aa, Artificial Sequence
  synthetic_VH-CDR2
  MOD_RES (1): Xaa is Gln, Phe, or Val
  MOD_RES (3): Xaa is Arg or Lys
  MOD_RES (4): Xaa is Asn, Ser, Gln, or Tyr
  MOD_RES (6): Xaa is Pro or Ala
  MOD_RES (8): Xaa is Asn or Gly
  MOD_RES (9): Xaa is Tyr, Gly, or Ser
  MOD_RES (10): Xaa is Glu or Thr
  MOD_RES (11): Xaa is Thr or Lys
  MOD_RES (12): Xaa is Tyr or Glu
  MOD_RES (14): Xaa is Ser, Ala, or Val
  MOD_RES (15): Xaa is Asn, Gln, or Ala
XIXXKXYXXXXXYXXSVKG

SEQ ID NO: 8 - protein, 19 aa, Artificial Sequence
  synthetic_VH-CDR2
QIRNKPYNYETYYSNSVKG

SEQ ID NO: 9 - protein, 19 aa, Artificial Sequence
  synthetic_VH-CDR2
QIRNKPYNYETYYSQSVKG

SEQ ID NO: 10 - protein, 19 aa, Artificial Sequence
  synthetic_VH-CDR2
QIRSKPYNYETYYAASVKG

SEQ ID NO: 11 - protein, 19 aa, Artificial Sequence
  synthetic_VH-CDR2
FIRSKAYGGTTEYAASVKG

SEQ ID NO: 12 - protein, 19 aa, Artificial Sequence
  synthetic_VH-CDR2
QIKQKPYNYEKYYVQSVKG

SEQ ID NO: 13 - protein, 19 aa, Artificial Sequence
  synthetic_VH-CDR2
QIKQKPYGGEKYYVQSVKG

SEQ ID NO: 14 - protein, 19 aa, Artificial Sequence
  synthetic_VH-CDR2
QIRNKPYNYEKYYAQSVKG

SEQ ID NO: 15 - protein, 19 aa, Artificial Sequence
  synthetic_VH-CDR2
VIRYKPYGSEKYYAQSVKG

SEQ ID NO: 16 - protein, 12 aa, Artificial Sequence
  synthetic_VH-CDR3
  MOD_RES (10): Xaa is Met or Phe
AMITSDGYAXDY

SEQ ID NO: 17 - protein, 12 aa, Artificial Sequence
  synthetic_VH-CDR3
AMITSDGYAMDY

SEQ ID NO: 18 - protein, 12 aa, Artificial Sequence
  synthetic_VH-CDR3
AMITSDGYAFDY

SEQ ID NO: 19 - protein, 17 aa, Artificial Sequence
  synthetic_VL-CDR1
  MOD_RES (1): Xaa is Lys or Arg
  MOD_RES (2): Xaa is Ser or Ala
  MOD_RES (6): Xaa is Leu or Val
  MOD_RES (8): Xaa is Leu, Tyr, or His
  MOD_RES (11): Xaa is Asn or Ser
  MOD_RES (12): Xaa is Gln or Gly
  MOD_RES (13): Xaa is Lys or Tyr
XXSQSXLXSSXXXNTLA

SEQ ID NO: 20 - protein, 17 aa, Artificial Sequence
  synthetic_VL-CDR1
KSSQSLLLSSNQKNYLA

SEQ ID NO: 21 - protein, 17 aa, Artificial Sequence
  synthetic_VL-CDR1
KSSQSVLLSSNQKNYLA

SEQ ID NO: 22 - protein, 17 aa, Artificial Sequence
  synthetic_VL-CDR1
KSSQSVLYSSNQKNYLA

SEQ ID NO: 23 - protein, 17 aa, Artificial Sequence
  synthetic_VL-CDR1
RSSQSLLLSSNQKNYLA

SEQ ID NO: 24 - protein, 17 aa, Artificial Sequence
  synthetic_VL-CDR1
RASQSVLLSSNQKNYLA

SEQ ID NO: 25 - protein, 17 aa, Artificial Sequence
  synthetic_VL-CDR1
RASQSVLLSSSQKNYLA

SEQ ID NO: 26 - protein, 17 aa, Artificial Sequence
  synthetic_VL-CDR1
RSSQSLLHSSNGYNYLA

SEQ ID NO: 27 - protein, 7 aa, Artificial Sequence
  synthetic_VL-CDR2
  MOD_RES (2): Xaa is Ala or Gly
  MOD_RES (4): Xaa is Thr or Ser
  MOD_RES (6): Xaa is Glu or Ala
  MOD_RES (7): Xaa is Ser or Thr
WXSXRXX

SEQ ID NO: 28 - protein, 7 aa, Artificial Sequence
  synthetic_VL-CDR2
WASTRES

SEQ ID NO: 29 - protein, 7 aa, Artificial Sequence
  synthetic_VL-CDR2
WASSRET

SEQ ID NO: 30 - protein, 7 aa, Artificial Sequence
  synthetic_VL-CDR2
WASSRAT

SEQ ID NO: 31 - protein, 7 aa, Artificial Sequence
  synthetic_VL-CDR2
WGSTRES

SEQ ID NO: 32 - protein, 7 aa, Artificial Sequence
  synthetic_VL-CDR2
WGSTRAS

SEQ ID NO: 33 - protein, 9 aa, Artificial Sequence
  synthetic_VL-CDR3
  MOD_RES (3): Xaa is Cys or Ser
  MOD_RES (5): Xaa is Ser or Gln
  MOD_RES (6): Xaa is Tyr, Thr, or Ser
  MOD_RES (8): Xaa is Leu or Tyr
QQXFXXPXT

SEQ ID NO: 34 - protein, 9 aa, Artificial Sequence
  synthetic_VL-CDR3
QQCFSYPLT

SEQ ID NO: 35 - protein, 9 aa, Artificial Sequence
  synthetic_VL-CDR3
QQSFSYPLT

SEQ ID NO: 36 - protein, 9 aa, Artificial Sequence
  synthetic_VL-CDR3
QQSFSTPYT

SEQ ID NO: 37 - protein, 9 aa, Artificial Sequence
  synthetic_VL-CDR3
QQSFSSPYT

SEQ ID NO: 38 - protein, 9 aa, Artificial Sequence
  synthetic_VL-CDR3
QQSFQTPYT

SEQ ID NO: 39 - protein, 30 aa, Artificial Sequence
  synthetic_VH-FR1
EVKVDETGGGLVQPGRPMKLSCVVSGITFS

SEQ ID NO: 40 - protein, 30 aa, Artificial Sequence
  synthetic_VH-FR1
EVKVVESGGGLVQPGRSLRLSCTASGITFS

SEQ ID NO: 41 - protein, 30 aa, Artificial Sequence
  synthetic_VH-FR1
EVQLVESGGGLVQPGRSLRLSCTASGITFG

SEQ ID NO: 42 - protein, 30 aa, Artificial Sequence
  synthetic_VH-FR1
EVQLVESGGGLVQPGRSLRLSCTASGFTFG

SEQ ID NO: 43 - protein, 30 aa, Artificial Sequence
  synthetic_VH-FR1
EVKVVESGGGLVQPGGSLRLSCAASGITFS

SEQ ID NO: 44 - protein, 30 aa, Artificial Sequence
  synthetic_VH-FR1
EVQLVESGGGLVQPGGSLRLSCAASGITFS

SEQ ID NO: 45 - protein, 30 aa, Artificial Sequence
  synthetic_VH-FR1
EVQLVESGGGLVQPGGSLRLSCAASGFTFS

SEQ ID NO: 46 - protein, 30 aa, Artificial Sequence
  synthetic_VH-FR1
QVKVVESGGGVVQPGRSLRLSCAASGITFS

SEQ ID NO: 47 - protein, 30 aa, Artificial Sequence
  synthetic_VH-FR1
QVQLVESGGGVVQPGRSLRLSCAASGITFS

SEQ ID NO: 48 - protein, 30 aa, Artificial Sequence
  synthetic_VH-FR1
QVQLVESGGGVVQPGRSLRLSCAASGFTFS

SEQ ID NO: 49 - protein, 14 aa, Artificial Sequence
  synthetic_VH-FR2
WVRQSPEKGLEWVA

SEQ ID NO: 50 - protein, 14 aa, Artificial Sequence
  synthetic_VH-FR2
WVRQAPGKGLEWVG

SEQ ID NO: 51 - protein, 14 aa, Artificial Sequence
  synthetic_VH-FR2
WVRQAPGKGLEWVA

SEQ ID NO: 52 - protein, 32 aa, Artificial Sequence
  synthetic_VH-FR3
RFTISRDDSKSSVYLQMNNLRAEDMGIYYCTW

SEQ ID NO: 53 - protein, 32 aa, Artificial Sequence
  synthetic_VH-FR3
RFTISRDDSKSIAYLQMSSLKTEDTAVYYCTW

SEQ ID NO: 54 - protein, 32 aa, Artificial Sequence
  synthetic_VH-FR3
RFTISRDDAKSSVYLQMSSLRAEDTAVYYCTW

SEQ ID NO: 55 - protein, 32 aa, Artificial Sequence
  synthetic_VH-FR3
RFTISRDDAKSSLYLQMSSLRAEDTAVYYCAW

SEQ ID NO: 56 - protein, 32 aa, Artificial Sequence
  synthetic_VH-FR3
RFTISRDDSKSTVYLQMSSLRAEDTAVYYCTW

SEQ ID NO: 57 - protein, 32 aa, Artificial Sequence
  synthetic_VH-FR3
RFTISRDDSKSTLYLQMSSLRAEDTAVYYCAW

SEQ ID NO: 58 - protein, 11 aa, Artificial Sequence
  synthetic_VH-FR4
WGQGTSVTVSS

SEQ ID NO: 59 - protein, 11 aa, Artificial Sequence
  synthetic_VH-FR4
WGQGTLVTVSS

SEQ ID NO: 60 - protein, 23 aa, Artificial Sequence
  synthetic_VL-FR1
DIVMSQSPSSLAVSVGEKVTLIC

SEQ ID NO: 61 - protein, 23 aa, Artificial Sequence
  synthetic_VL-FR1
DIVMTQSPDSLAVSLGERATISC

SEQ ID NO: 62 - protein, 23 aa, Artificial Sequence
  synthetic_VL-FR1
EIVMTQSPGTLSLSPGERATLSC

SEQ ID NO: 63 - protein, 23 aa, Artificial Sequence
  synthetic_VL-FR1
EIVLTQSPGTLSLSPGERATLSC

SEQ ID NO: 64 - protein, 23 aa, Artificial Sequence
  synthetic_VL-FR1
DIVMTQSPLSLPVTPGEPASISC

SEQ ID NO: 65 - protein, 15 aa, Artificial Sequence
  synthetic_VL-FR2
WYQQKPGQSPKLLIY

SEQ ID NO: 66 - protein, 15 aa, Artificial Sequence
  synthetic_VL-FR2
WYQQKPGQPPKLLIY

SEQ ID NO: 67 - protein, 15 aa, Artificial Sequence
  synthetic_VL-FR2
WYQQKPGQAPRLLIY

SEQ ID NO: 68 - protein, 15 aa, Artificial Sequence
  synthetic_VL-FR2
WYLQKPGQSPQLLIY

SEQ ID NO: 69 - protein, 32 aa, Artificial Sequence
  synthetic_VL-FR3
GVPDRFTGSGSGTDFTLTINSVKAEDLAVYYC

SEQ ID NO: 70 - protein, 32 aa, Artificial Sequence
  synthetic_VL-FR3
GVPDRFSGSGSGTEFTLTISSVQAEDVAVYYC

SEQ ID NO: 71 - protein, 32 aa, Artificial Sequence
  synthetic_VL-FR3
GVPDRFSGSGSGTEFTLTISSLQAEDVAVYYC

SEQ ID NO: 72 - protein, 32 aa, Artificial Sequence
  synthetic_VL-FR3
GIPDRFSGSGSGTDFTLTISRVEPEDFAVYYC

SEQ ID NO: 73 - protein, 32 aa, Artificial Sequence
  synthetic_VL-FR3
GIPDRFSGSGSGTDFTLTISRLEPEDFAVYYC

SEQ ID NO: 74 - protein, 31 aa, Artificial Sequence
  synthetic_VL-FR3
VPDRFSGSGSGTDFTLKISRVEAEDVGVYYC

SEQ ID NO: 75 - protein, 10 aa, Artificial Sequence
  synthetic_VL-FR4
FGAGTKLELK

SEQ ID NO: 76 - protein, 10 aa, Artificial Sequence
  synthetic_VL-FR4
FGQGTKLEIK

SEQ ID NO: 77 - protein, 123 aa, Artificial Sequence
  synthetic_VH-chimeric
EVKVDETGGGLVQPGRPMKLSCVVSGITFSDYWMNWVRQSPEKGLEWVAQIRNKPYNYETYYSNSVKGRFTISRDDSKSSVYLQMNNLRAEDMGIYYCTWAMITSDGYAMDYWGQGTSVTVSS

SEQ ID NO: 78 - protein, 123 aa, Artificial Sequence
  synthetic_VH1 (MP1-H349-V1)
EVKVVESGGGLVQPGRSLRLSCTASGITFSDYWMNWVRQAPGKGLEWVGQIRNKPYNYETYYSQSVKGRFTISRDDSKSIAYLQMSSLKTEDTAVYYCTWAMITSDGYAMDYWGQGTLVTVSS

SEQ ID NO: 79 - protein, 123 aa, Artificial Sequence
  synthetic_VH2 (MP1-H349-V2)
EVQLVESGGGLVQPGRSLRLSCTASGITFGDYWMNWVRQAPGKGLEWVGQIRSKPYNYETYYAASVKGRFTISRDDSKSIAYLQMSSLKTEDTAVYYCTWAMITSDGYAMDYWGQGTLVTVSS

SEQ ID NO: 80 - protein, 123 aa, Artificial Sequence
  synthetic_VH3 (MP1-H349-V3)
EVQLVESGGGLVQPGRSLRLSCTASGFTFGDYWMSWVRQAPGKGLEWVGFIRSKAYGGTTEYAASVKGRFTISRDDSKSIAYLQMSSLKTEDTAVYYCTWAMITSDGYAFDYWGQGTLVTVSS

SEQ ID NO: 81 - protein, 123 aa, Artificial Sequence
  synthetic_VH4 (MP1-H37-V1)
EVKVVESGGGLVQPGGSLRLSCAASGITFSDYWMNWVRQAPGKGLEWVAQIRNKPYNYETYYSNSVKGRFTISRDDAKSSVYLQMSSLRAEDTAVYYCTWAMITSDGYAMDYWGQGTLVTVSS

SEQ ID NO: 82 - protein, 123 aa, Artificial Sequence
  synthetic_VH5 (MP1-H37-V2)
EVQLVESGGGLVQPGGSLRLSCAASGITFSSYWMNWVRQAPGKGLEWVAQIKQKPYNYEKYYVQSVKGRFTISRDDAKSSLYLQMSSLRAEDTAVYYCAWAMITSDGYAMDYWGQGTLVTVSS

SEQ ID NO: 83 - protein, 123 aa, Artificial Sequence
  synthetic_VH6 (MP1-H37-V3)
EVQLVESGGGLVQPGGSLRLSCAASGFTFSSYWMSWVRQAPGKGLEWVAQIKQKPYGGEKYYVQSVKGRFTISRDDAKSSLYLQMSSLRAEDTAVYYCAWAMITSDGYAFDYWGQGTLVTVSS

SEQ ID NO: 84 - protein, 123 aa, Artificial Sequence
  synthetic_VH7 (MP1-H333-V1)
QVKVVESGGGVVQPGRSLRLSCAASGITFSDYWMNWVRQAPGKGLEWVAQIRNKPYNYETYYSNSVKGRFTISRDDSKSTVYLQMSSLRAEDTAVYYCTWAMITSDGYAMDYWGQGTLVTVSS

SEQ ID NO: 85 - protein, 123 aa, Artificial Sequence
  synthetic_VH8 (MP1-H333-V2)
QVQLVESGGGVVQPGRSLRLSCAASGITFSSYWMNWVRQAPGKGLEWVAQIRNKPYNYEKYYAQSVKGRFTISRDDSKSTLYLQMSSLRAEDTAVYYCAWAMITSDGYAMDYWGQGTLVTVSS

SEQ ID NO: 86 - protein, 123 aa, Artificial Sequence
  synthetic_VH9 (MP1-H333-V3)
QVQLVESGGGVVQPGRSLRLSCAASGFTFSSYWMHWVRQAPGKGLEWVAVIRYKPYGSEKYYAQSVKGRFTISRDDSKSTLYLQMSSLRAEDTAVYYCAWAMITSDGYAFDYWGQGTLVTVSS

SEQ ID NO: 87 - protein, 113 aa, Artificial Sequence
  synthetic_VL-chimeric
DIVMSQSPSSLAVSVGEKVTLICKSSQSLLLSSNQKNYLAWYQQKPGQSPKLLIYWASTRESGVPDRFTGSGSGTDFTLTINSVKAEDLAVYYCQQCFSYPLTFGAGTKLELK

SEQ ID NO: 88 - protein, 113 aa, Artificial Sequence
  synthetic_VL1 (MP1-L41-V1)
DIVMTQSPDSLAVSLGERATISCKSSQSLLLSSNQKNYLAWYQQKPGQPPKLLIYWASTRESGVPDRFSGSGSGTEFTLTISSVQAEDVAVYYCQQCFSYPLTFGQGTKLEIK

SEQ ID NO: 89 - protein, 113 aa, Artificial Sequence
  synthetic_VL2 (MP1-L41-V2)
DIVMTQSPDSLAVSLGERATISCKSSQSVLLSSNQKNYLAWYQQKPGQPPKLLIYWASTRESGVPDRFSGSGSGTEFTLTISSLQAEDVAVYYCQQSFSYPLTFGQGTKLEIK

SEQ ID NO: 90 - protein, 113 aa, Artificial Sequence
  synthetic_VL3 (MP1-L41-V3)
DIVMTQSPDSLAVSLGERATISCKSSQSVLYSSNQKNYLAWYQQKPGQPPKLLIYWASTRESGVPDRFSGSGSGTEFTLTISSLQAEDVAVYYCQQSFSTPYTFGQGTKLEIK

SEQ ID NO: 91 - protein, 113 aa, Artificial Sequence
  synthetic_VL4 (MP1-L320-V1)
EIVMTQSPGTLSLSPGERATLSCRSSQSLLLSSNQKNYLAWYQQKPGQAPRLLIYWASTRESGIPDRFSGSGSGTDFTLTISRVEPEDFAVYYCQQCFSYPLTFGQGTKLEIK

SEQ ID NO: 92 - protein, 113 aa, Artificial Sequence
  synthetic_VL5 (MP1-L320-V2)
EIVLTQSPGTLSLSPGERATLSCRASQSVLLSSNQKNYLAWYQQKPGQAPRLLIYWASSRETGIPDRFSGSGSGTDFTLTISRLEPEDFAVYYCQQSFSYPLTFGQGTKLEIK

SEQ ID NO: 93 - protein, 113 aa, Artificial Sequence
  synthetic_VL6 (MP1-L320-V3)
EIVLTQSPGTLSLSPGERATLSCRASQSVLLSSSQKNYLAWYQQKPGQAPRLLIYWASSRATGIPDRFSGSGSGTDFTLTISRLEPEDFAVYYCQQSFSSPYTFGQGTKLEIK

SEQ ID NO: 94 - protein, 113 aa, Artificial Sequence
  synthetic_VL7 (MP1-L228-V1)
DIVMTQSPLSLPVTPGEPASISCRSSQSLLLSSNQKNYLAWYLQKPGQSPQLLIYWASTRESGVPDRFSGSGSGTDFTLKISRVEAEDVGVYYCQQCFSYPLTFGQGTKLEIK

SEQ ID NO: 95 - protein, 113 aa, Artificial Sequence
  synthetic_VL8 (MP1-L228-V2)
DIVMTQSPLSLPVTPGEPASISCRSSQSLLLSSNQKNYLAWYLQKPGQSPQLLIYWGSTRESGVPDRFSGSGSGTDFTLKISRVEAEDVGVYYCQQSFSYPLTFGQGTKLEIK

SEQ ID NO: 96 - protein, 113 aa, Artificial Sequence
  synthetic_VL9 (MP1-L228-V3)
DIVMTQSPLSLPVTPGEPASISCRSSQSLLHSSNGYNYLAWYLQKPGQSPQLLIYWGSTRASGVPDRFSGSGSGTDFTLKISRVEAEDVGVYYCQQSFQTPYTFGQGTKLEIK

SEQ ID NO: 97 - protein, 8 aa, Artificial Sequence
  synthetic_OKT3 VH-CDR1
GYTFTRYT

SEQ ID NO: 98 - protein, 8 aa, Artificial Sequence
  synthetic_OKT3 VH-CDR2
INPSRGYT

SEQ ID NO: 99 - protein, 12 aa, Artificial Sequence
  synthetic_OKT3 VH-CDR3
ARYYDDHYSLDY

SEQ ID NO: 100 - protein, 7 aa, Artificial Sequence
  synthetic_OKT3 VL-CDR1
ASSSVSY

SEQ ID NO: 101 - protein, 3 aa, Artificial Sequence
  synthetic_OKT3 VL-CDR2
DTS

SEQ ID NO: 102 - protein, 9 aa, Artificial Sequence
  synthetic_OKT3 VL-CDR3
QQWSSNPFT

SEQ ID NO: 103 - protein, 119 aa, Artificial Sequence
  synthetic_OKT3 VH
QVQLVQSGGGVVQPGRSLRLSCKASGYTFTRYTMHWVRQAPGKGLEWIGYINPSRGYTNYNQKVKDRFTISRDNSKNTAFLQMDSLRPEDTGVYFCARYYDDHYSLDYWGQGTPVTVSS

SEQ ID NO: 104 - protein, 106 aa, Artificial Sequence [sequence omitted]

SEQ ID NO: 105 - protein, 107 aa, Artificial Sequence
  synthetic_OKT3 VL
DIQMTQSPSSLSASVGDRVTITCSASSSVSYMNWYQQTPGKAPKRWIYDTSKLASGVPSRFSGSGSGTDYTFTISSLQPEDIATYYCQQWSSNPFTFGQGTKLQITR

SEQ ID NO: 106 - protein, 246 aa, Artificial Sequence
  synthetic_OKT3 scFv
QVQLVQSGGGVVQPGRSLRLSCKASGYTFTRYTMHWVRQAPGKCLEWIGYINPSRGYTNYNQKVKDRFTISRDNSKNTAFLQMDSLRPEDTGVYFCARYYDDHYSLDYWGQGTPVTVSSGGGSGGGSGGGSGGGSGGGSDIQMTQSPSSLSASVGDRVTITCSASSSVSYMNWYQQTPGKAPKRWIYDTSKLASGVPSRFSGSGSGTDYTFTISSLQPEDIATYYCQQWSSNPFTFGQCTKLQITR

SEQ ID NO: 107 - protein, 11 aa, Artificial Sequence
  synthetic_MUC1 antigen band
QGGFLGLSNIK

SEQ ID NO: 108 - protein, 255 aa, Artificial Sequence
  synthetic_MUC1 isoform 2 (P15941-2) aa 895~1264
PAPGSTAPPAHGVTSAPDTRPAPGSTAPPAHGVTSAPDTRPAPGSTAPPAHGVTSAPDNRPALGSTAPPVHNVTSASGSASGSASTLVHNGTSARATTTPASKSTPFSIPSHHSDTPTTLASHSTKTDASSTHHSSVPPLTSSNHSTSPQLSTGVSFFFLSFHISNLQFNSSLEDPSTDYYQELQRDISEMFLQIYKQGGFLGLSNIKFRPGSVVVQLTLAFREGTINVHDVETQFNQYKTEAASRYNLTISDVS

SEQ ID NO: 109 - protein, 7 aa, Artificial Sequence
  synthetic_MUC1 epitope
PAHGVTS

SEQ ID NO: 110 - protein, 220 aa, Artificial Sequence
  synthetic_VL4 light chain
EIVMTQSPGTLSLSPGERATLSCRSSQSLLLSSNQKNYLAWYQQKPGQAPRLLIYWASTRESGIPDRFSGSGSGTDFTLTISRVEPEDFAVYYCQQCFSYPLTFGQGTKLEIKRTVAAPSVFIFPPSDEQLKSGTASVVCLLNNFYPREAKVQWKVDNALQSGNSQESVTEQDSKDSTYSLSSTLTLSKADYEKHKVYACEVTHQGLSSPVTKSFNRGEC

SEQ ID NO: 111 - protein, 220 aa, Artificial Sequence
  synthetic_VL5 light chain
EIVLTQSPGTLSLSPGERATLSCRASQSVLLSSNQKNYLAWYQQKPGQAPRLLIYWASSRETGIPDRFSGSGSGTDFTLTISRLEPEDFAVYYCQQSFSYPLTFGQGTKLEIKRTVAAPSVFIFPPSDEQLKSGTASVVCLLNNFYPREAKVQWKVDNALQSGNSQESVTEQDSKDSTYSLSSTLTLSKADYEKHKVYACEVTHQGLSSPVTKSFNRGEC

SEQ ID NO: 112 - protein, 255 aa, Artificial Sequence
  synthetic_LCC version humanized MP1 Light chain #4-OKT3scFv
EIVMTQSPGTLSLSPGERATLSCRSSQSLLLSSNQKNYLAWYQQKPGQAPRLLIYWASTRESGIPDRFSGSGSGTDFTLTISRVEPEDFAVYYCQQCFSYPLTFGQGTKLEIKRTVAAPSVFIFPPSDEQLKSGTASVVCLLNNFYPREAKVQWKVDNALQSGNSQESVTEQDSKDSTYSLSSTLTLSKADYEKHKVYACEVTHQGLSSPVTKSFNRGECGGGSGGGSGGGSQVQLVQSGGGVVQPGRSLRLSCK

SEQ ID NO: 113 - protein, 255 aa, Artificial Sequence
  synthetic_LCC version humanized MP1 Light chain #5-OKT3scFv
EIVLTQSPGTLSLSPGERATLSCRASQSVLLSSNQKNYLAWYQQKPGQAPRLLIYWASSRETGIPDRFSGSGSGTDFTLTISRLEPEDFAVYYCQQSFSYPLTFGQGTKLEIKRTVAAPSVFIFPPSDEQLKSGTASVVCLLNNFYPREAKVQWKVDNALQSGNSQESVTEQDSKDSTYSLSSTLTLSKADYEKHKVYACEVTHQGLSSPVTKSFNRGECGGGSGGGSGGGSQVQLVQSGGGVVQPGRSLRLSCK

SEQ ID NO: 114 - protein, 255 aa, Artificial Sequence
  synthetic_LCN version humanized MP1 Light chain #4-OKT3scFv
QVQLVQSGGGVVQPGRSLRLSCKASGYTFTRYTMHWVRQAPGKCLEWIGYINPSRGYTNYNQKVKDRFTISRDNSKNTAFLQMDSLRPEDTGVYFCARYYDDHYSLDYWGQGTPVTVSSGGGSGGGSGGGSGGGSGGGSDIQMTQSPSSLSASVGDRVTITCSASSSVSYMNWYQQTPGKAPKRWIYDTSKLASGVPSRFSGSGSGTDYTFTISSLQPEDIATYYCQQWSSNPFTFGQCTKLQITRGGGSGGGSG

SEQ ID NO: 115 - protein, 255 aa, Artificial Sequence; identical to SEQ ID NO: 114
  synthetic_LCN version humanized MP1 Light chain #5-OKT3scFv